European Patent Application EP 4 582 457 A1, published July 9, 2025. Title: Artificial protein and pharmaceutical composition. Applicant: MiraBiologics Inc. The sequence listing filed with the application follows.

SEQUENCE LISTING (45 sequences)

SEQ ID NO: 1 - protein, 28 aa, synthetic construct
  REGION 1..6: note = X can be any amino acid. One or more X in this region may be deleted.
  REGION 23..28: note = X can be any amino acid. One or more X in this region may be deleted.
  SITE 8..9: note = X can be any amino acid.
  SITE 15..17: note = X can be any amino acid.
  SITE 19..22: note = X can be any amino acid.
XXXXXXYXXFYYNYXXXWXXXXXXXXXX

SEQ ID NO: 2 - protein, 208 aa, Homo sapiens
VFLFPPKPKDTLMISRTPEVTCVVVDVSHEDPEVKFNWYVDGVEVHNAKTKPREEQYNSTYRVVSVLTVLHQDWLNGKEYKCKVSNKALGAPIEKTISKAKGQPREPQVYTLPPSRDELTKNQVSLTCLVKGFYPSDIAVEWESNGQPENNYKTTPPVLDSDGSFFLYSKLTVDKSRWQQGNVFSCSVMHEALHNHYTQKSLSLSPGK

SEQ ID NO: 3 - protein, 227 aa, Homo sapiens
DKTHTCPPCPAPELLGGPSVFLFPPKPKDTLMISRTPEVTCVVVDVSHEDPEVKFNWYVDGVEVHNAKTKPREEQYNSTYRVVSVLTVLHQDWLNGKEYKCKVSNKALPAPIEKTISKAKGQPREPQVYTLPPSRDELTKNQVSLTCLVKGFYPSDIAVEWESNGQPENNYKTTPPVLDSDGSFFLYSKLTVDKSRWQQGNVFSCSVMHEALHNHYTQKSLSLSPGK

SEQ ID NO: 4 - protein, 208 aa, Homo sapiens
VFLFPPKPKDTLMISRTPEVTCVVVDVSHEDPEVKFNWYVDGVEVHNAKTKPREEQYNSTYRVVSVLTVLHQDWLNGKEYKCKVSNKALPAPIEKTISKAKGQPREPQVYTLPPSRDELTKNQVSLTCLVKGFYPSDIAVEWESNGQPENNYKTTPPVLDSDGSFFLYSKLTVDKSRWQQGNVFSCSVMHEALHNHYTQKSLSLSPGK

SEQ ID NO: 5 - protein, 5 aa, Homo sapiens
SHEDP

SEQ ID NO: 6 - protein, 4 aa, Homo sapiens
YNST

SEQ ID NO: 7 - protein, 7 aa, Homo sapiens
NKALPAP

SEQ ID NO: 8 - protein, 4 aa, Homo sapiens
VDGV

SEQ ID NO: 9 - protein, 4 aa, Homo sapiens
SDGS

SEQ ID NO: 10 - protein, 4 aa, Homo sapiens
TKNQ

SEQ ID NO: 11 - protein, 5 aa, Homo sapiens
QQGNV

SEQ ID NO: 12 - protein, 227 aa, Homo sapiens
DKTHTCPPCPAPEAAGGPSVFLFPPKPKDTLMISRTPEVTCVVVDVSHEDPEVKFNWYVDGVEVHNAKTKPREEQYNSTYRVVSVLTVLHQDWLNGKEYKCKVSNKALGAPIEKTISKAKGQPREPQVYTLPPSRDELTKNQVSLTCLVKGFYPSDIAVEWESNGQPENNYKTTPPVLDSDGSFFLYSKLTVDKSRWQQGNVFSCSVMHEALHNHYTQKSLSLSPGK

SEQ ID NO: 13 - protein, 248 aa, synthetic construct
DKTHTCPPCPAPEAAGGPSVFLFPPKPKDTLMISRTPEVTCVVVDVSHEDPEVKFNWYVDGVEVHNAKTKPREEQYNSTYRVVSVLTVLHQDWLNGKEYKCKVSNKALGAPIEKTISKAKGQPREPQVYTLPPSRDELTKNQVSLTCLVKGFYPSDIAVEWESSGGYPTFYYNYRSEWVLTSGGSGQPENNYKTTPPVLDSDGSFFLYSKLTVDKSRWQQGNVFSCSVMHEALHNHYTQKSLSLSPGK

SEQ ID NO: 14 - protein, 248 aa, synthetic construct
DKTHTCPPCPAPEAAGGPSVFLFPPKPKDTLMISRTPEVTCVVVDVSHEDPEVKFNWYVDGVEVHNAKTKPREEQYNSTYRVVSVLTVLHQDWLNGKEYKCKVSNKALGAPIEKTISKAKGQPREPQVYTLPPSRDELTKNQVSLTCLVKGFYPSDIAVEWESNGQPENNYKTTPPVLDSDGSFFLYSKLTVDKSRWQQSGGYPTFYYNYRSEWVLTSGGSNVFSCSVMHEALHNHYTQKSLSLSPGK

SEQ ID NO: 15 - protein, 248 aa, synthetic construct
DKTHTCPPCPAPELLGGPSVFLFPPKPKDTLMISRTPEVTCVVVDVSHEDPEVKFNWYVDGVEVHNAKTKPREEQYNSTYRVVSVLTVLHQDWLNGKEYKCKVSNKALPAPIEKTISKAKGQPREPQVYTLPPSRDELTKNQVSLTCLVKGFYPSDIAVEWESSGGYPTFYYNYRSEWVLTSGGSGQPENNYKTTPPVLDSDGSFFLYSKLTVDKSRWQQGNVFSCSVMHEALHNHYTQKSLSLSPGK

SEQ ID NO: 16 - protein, 248 aa, synthetic construct
DKTHTCPPCPAPELLGGPSVFLFPPKPKDTLMISRTPEVTCVVVDVSHEDPEVKFNWYVDGVEVHNAKTKPREEQYNSTYRVVSVLTVLHQDWLNGKEYKCKVSNKALPAPIEKTISKAKGQPREPQVYTLPPSRDELTKNQVSLTCLVKGFYPSDIAVEWESNGQPENNYKTTPPVLDSDGSFFLYSKLTVDKSRWQQSGGYPTFYYNYRSEWVLTSGGSNVFSCSVMHEALHNHYTQKSLSLSPGK

SEQ ID NO: 17 - protein, 22 aa, synthetic construct
SGGYPTFYYNYRSEWVLTSGGS

SEQ ID NO: 18 - protein, 15 aa, synthetic construct
YRQFNRRTHEVWNLD

SEQ ID NO: 19 - protein, 17 aa, synthetic construct
CYRQFNRRTHEVWNLDC

SEQ ID NO: 20 - protein, 13 aa, synthetic construct
WYYAWDQTYKAFP

SEQ ID NO: 21 - protein, 245 aa, synthetic construct
DKTHTCPPCPAPELLGGPSVFLFPPKPKDTLMISRTPEVTCVVVDVSHEDPEVKFNWYVDGVEVHNAKTKPREEQYNSTYRVVSVLTVLHQDWLNGKEYKCKVSNKALPAPIEKTISKAKGQPREPQVYTLPPSRDELTKNQVSLTCLVKGFYPSDIAVEWESGGYRQFNRRTHEVWNLDGGGQPENNYKTTPPVLDSDGSFFLYSKLTVDKSRWQQGNVFSCSVMHEALHNHYTQKSLSLSPGK

SEQ ID NO: 22 - protein, 245 aa, synthetic construct
DKTHTCPPCPAPELLGGPSVFLFPPKPKDTLMISRTPEVTCVVVDVSHEDPEVKFNWYVDGVEVHNAKTKPREEQYNSTYRVVSVLTVLHQDWLNGKEYKCKVSNKALPAPIEKTISKAKGQPREPQVYTLPPSRDELTKNQVSLTCLVKGFYPSDIAVEWESNGQPENNYKTTPPVLDSDGSFFLYSKLTVDKSRWQQGGYRQFNRRTHEVWNLDGGNVFSCSVMHEALHNHYTQKSLSLSPGK

SEQ ID NO: 23 - protein, 247 aa, synthetic construct
DKTHTCPPCPAPELLGGPSVFLFPPKPKDTLMISRTPEVTCVVVDVSHEDPEVKFNWYVDGVEVHNAKTKPREEQYNSTYRVVSVLTVLHQDWLNGKEYKCKVSNKALPAPIEKTISKAKGQPREPQVYTLPPSRDELTKNQVSLTCLVKGFYPSDIAVEWESGGCYRQFNRRTHEVWNLDCGGGQPENNYKTTPPVLDSDGSFFLYSKLTVDKSRWQQGNVFSCSVMHEALHNHYTQKSLSLSPGK

SEQ ID NO: 24 - protein, 247 aa, synthetic construct
DKTHTCPPCPAPELLGGPSVFLFPPKPKDTLMISRTPEVTCVVVDVSHEDPEVKFNWYVDGVEVHNAKTKPREEQYNSTYRVVSVLTVLHQDWLNGKEYKCKVSNKALPAPIEKTISKAKGQPREPQVYTLPPSRDELTKNQVSLTCLVKGFYPSDIAVEWESNGQPENNYKTTPPVLDSDGSFFLYSKLTVDKSRWQQGGCYRQFNRRTHEVWNLDCGGNVFSCSVMHEALHNHYTQKSLSLSPGK

SEQ ID NO: 25 - protein, 247 aa, synthetic construct
DKTHTCPPCPAPEAAGGPSVFLFPPKPKDTLMISRTPEVTCVVVDVSHEDPEVKFNWYVDGVEVHNAKTKPREEQYNSTYRVVSVLTVLHQDWLNGKEYKCKVSNKALGAPIEKTISKAKGQPREPQVYTLPPSRDELTKNQVSLTCLVKGFYPSDIAVEWESNGQPENNYKTTPPVLDSDGSFFLYSKLTVDKSRWQQGGCYRQFNRRTHEVWNLDCGGNVFSCSVMHEALHNHYTQKSLSLSPGK

SEQ ID NO: 26 - protein, 243 aa, synthetic construct
DKTHTCPPCPAPELLGGPSVFLFPPKPKDTLMISRTPEVTCVVVDVSHEDPEVKFNWYVDGVEVHNAKTKPREEQYNSTYRVVSVLTVLHQDWLNGKEYKCKVSNKALPAPIEKTISKAKGQPREPQVYTLPPSRDELTKNQVSLTCLVKGFYPSDIAVEWESGGWYYAWDQTYKAFPGGGQPENNYKTTPPVLDSDGSFFLYSKLTVDKSRWQQGNVFSCSVMHEALHNHYTQKSLSLSPGK

SEQ ID NO: 27 - protein, 243 aa, synthetic construct
DKTHTCPPCPAPELLGGPSVFLFPPKPKDTLMISRTPEVTCVVVDVSHEDPEVKFNWYVDGVEVHNAKTKPREEQYNSTYRVVSVLTVLHQDWLNGKEYKCKVSNKALPAPIEKTISKAKGQPREPQVYTLPPSRDELTKNQVSLTCLVKGFYPSDIAVEWESNGQPENNYKTTPPVLDSDGSFFLYSKLTVDKSRWQQGGWYYAWDQTYKAFPGGNVFSCSVMHEALHNHYTQKSLSLSPGK

SEQ ID NO: 28 - protein, 28 aa, synthetic construct
  REGION 1..6: note = X can be any amino acid. One or more X in this region may be deleted.
  REGION 23..28: note = X can be any amino acid. One or more X in this region may be deleted.
XXXXXXYPTFYYNYRSEWVLTSXXXXXX

SEQ ID NO: 29 - protein, 22 aa, synthetic construct
  SITE 5..6: note = X can be any amino acid.
  SITE 12..14: note = X can be any amino acid.
  SITE 16..19: note = X can be any amino acid.
SGGYXXFYYNYXXXWXXXXGGS

SEQ ID NO: 30 - protein, 16 aa, synthetic construct
YPTFYYNYRSEWVLTS

SEQ ID NO: 31 - protein, 16 aa, synthetic construct
YATFYYNYRSEWVLTS

SEQ ID NO: 32 - protein, 16 aa, synthetic construct
YPAFYYNYRSEWVLTS

SEQ ID NO: 33 - protein, 16 aa, synthetic construct
YPTAYYNYRSEWVLTS

SEQ ID NO: 34 - protein, 16 aa, synthetic construct
YPTFAYNYRSEWVLTS

SEQ ID NO: 35 - protein, 16 aa, synthetic construct
YPTFYANYRSEWVLTS

SEQ ID NO: 36 - protein, 16 aa, synthetic construct
YPTFYYAYRSEWVLTS

SEQ ID NO: 37 - protein, 16 aa, synthetic construct
YPTFYYNARSEWVLTS

SEQ ID NO: 38 - protein, 16 aa, synthetic construct
YPTFYYNYASEWVLTS

SEQ ID NO: 39 - protein, 16 aa, synthetic construct
YPTFYYNYRAEWVLTS

SEQ ID NO: 40 - protein, 16 aa, synthetic construct
YPTFYYNYRSAWVLTS

SEQ ID NO: 41 - protein, 16 aa, synthetic construct
YPTFYYNYRSEAVLTS

SEQ ID NO: 42 - protein, 16 aa, synthetic construct
YPTFYYNYRSEWALTS

SEQ ID NO: 43 - protein, 16 aa, synthetic construct
YPTFYYNYRSEWVATS

SEQ ID NO: 44 - protein, 16 aa, synthetic construct
YPTFYYNYRSEWVLAS

SEQ ID NO: 45 - protein, 16 aa, synthetic construct
YPTFYYNYRSEWVLTA